European Patent Specification EP 3 848 457 B1, published August 13, 2025. Title: MULTIPLE LIGASE COMPOSITIONS, SYSTEMS, AND METHODS. Applicant: RGENE, INC. The sequence listing filed with the application follows.

SEQUENCE LISTING (24 sequences)

SEQ ID NO: 1 - protein, 487 aa, Artificial sequence
  Synthetic
MILKILNEIASIGSTKQKQAILEKNKDNELLKRVYRLTYSRGLQYYIKKWPKPGIATQSFGMLTLTDMLDFIEFTLATRKLTGNAAIEELTGYITDGKKDDVEVLRRVMMRDLECGASVSIANKVWPGLIPEQPQMLASSYDEKGINKNIKFPAFAQLSADGARCFAEVRGDELDDVRLLSRAGNEYLGLDLLKEELIKMTAEARQIHPEGVLIDGELVYHEQVKKEPEGLDFLFDAYPENSKAKEFAEVAESRTASNGIANKSLKGTISEKEAQCMKFQVWDYVPLVEIYSLPAFRLKYDVRFSKLEQMTSGYDKVILIENQVVNNLDEAKVIYKKYIDQGLEGIILKNIDGLWENARSKNLYKFKEVIDVDLKIVGIYPHRKDPTKAGGFILESECGKIKVNAGSGLKDKAGVKSHELDRTRIMENQNYYIGKILECECNGWLKSDGRTDYVKLFLPIAIRLREDKTKANTFEDVFGDFHEVTGL

SEQ ID NO: 2 - protein, 487 aa, Artificial sequence
  Synthetic
MILKILNEIASIGSTKQKQAILEKNKDNELLKRVYRLTYSRGLQYYIKKWPKPGIATQSFGMLTLTDMLDFIEFTLATRKLTGNAAIEELTGYITDGKKDDVEVLRRVMMRDLECGASVSIANKVWPGLIPEQPQMLASSYDEKGINKNIKFPAFAQLCADGARCFAEVRGDELDDVRLLSRAGNEYLGLDLLKEELIKMTAEARQIHPEGVLIDGELVYHEQVKKEPEGLDFLFDAYPENSKAKEFAEVAESRTASNGIANKSLKGTISEKEAQCMKFQVWDYVPLVEIYSLPAFRLKYDVRFSKLEQMTSGYDKVILIENQVVNNLDEAKVIYKKYIDQGLEGIILKNIDGLWENARSKNLYKFKEVIDVDLKIVGIYPHRKDPTKAGGFILESECGKIKVNAGSGLKDKAGVKSHELDRTRIMENQNYYIGKILECECNGWLKSDGRTDYVKLFLPIAIRLREDKTKANTFEDVFGDFHEVTGL

SEQ ID NO: 3 - protein, 487 aa, Artificial sequence
  Synthetic
MILKILNEIASIGSTKQKQAILEKNKDNELLKRVYRLTYSRGLQYYIKKWPKPGIATQSFGMLTLTDMLDFIEFTLATRKLTGNAAIEELTGYITDGKKDDVEVLRRVMMRDLECGASVSIANKVWPGLIPEQPQMLASSYDEKGINKNIKFPAFAQLAADGARCFAEVRGDELDDVRLLSRAGNEYLGLDLLKEELIKMTAEARQIHPEGVLIDGELVYHEQVKKEPEGLDFLFDAYPENSKAKEFAEVAESRTASNGIANKSLKGTISEKEAQCMKFQVWDYVPLVEIYSLPAFRLKYDVRFSKLEQMTSGYDKVILIENQVVNNLDEAKVIYKKYIDQGLEGIILKNIDGLWENARSKNLYKFKEVIDVDLKIVGIYPHRKDPTKAGGFILESECGKIKVNAGSGLKDKAGVKSHELDRTRIMENQNYYIGKILECECNGWLKSDGRTDYVKLFLPIAIRLREDKTKANTFEDVFGDFHEVTGL

SEQ ID NO: 4 - DNA, 64 bp, Artificial sequence
  Synthetic
gatcggaagagcacacgtctgaactccagtcuacactctttccctacacgacgctcttccgatc

SEQ ID NO: 5 - protein, 4 aa, Artificial sequence
  Synthetic
  MISC_FEATURE (2)..(2): Xaa=any amino acid
  MISC_FEATURE (3)..(3): Xaa= D or N
GXXG

SEQ ID NO: 6 - protein, 4 aa, Artificial sequence
  Synthetic
  MISC_FEATURE (2)..(2): Xaa=any amino acid
  MISC_FEATURE (3)..(3): Xaa=D or N
PXXG

SEQ ID NO: 7 - protein, 4 aa, Artificial sequence
  Synthetic
  MISC_FEATURE (2)..(2): Xaa=any amino acid
  MISC_FEATURE (3)..(3): Xaa=D or N
AXXG

SEQ ID NO: 8 - protein, 4 aa, Artificial sequence
  Synthetic
  MISC_FEATURE (2)..(2): Xaa=any amino acid
  MISC_FEATURE (3)..(3): Xaa=D or N
VXXG

SEQ ID NO: 9 - protein, 4 aa, Artificial sequence
  Synthetic
  MISC_FEATURE (2)..(2): Xaa=any amino acid
  MISC_FEATURE (3)..(3): Xaa=D or N
LXXG

SEQ ID NO: 10 - protein, 4 aa, Artificial sequence
  Synthetic
  MISC_FEATURE (2)..(2): Xaa=any amino acid
  MISC_FEATURE (3)..(3): Xaa=D or N
IXXG

SEQ ID NO: 11 - protein, 4 aa, Artificial sequence
  Synthetic
  MISC_FEATURE (2)..(2): Xaa=any amino acid
  MISC_FEATURE (3)..(3): Xaa=D or N
MXXG

SEQ ID NO: 12 - protein, 4 aa, Artificial sequence
  Synthetic
  MISC_FEATURE (2)..(2): Xaa=any amino acid
  MISC_FEATURE (3)..(3): Xaa=D or N
CXXG

SEQ ID NO: 13 - protein, 4 aa, Artificial sequence
  Synthetic
  MISC_FEATURE (2)..(2): Xaa=any amino acid
  MISC_FEATURE (3)..(3): Xaa=D or N
FXXG

SEQ ID NO: 14 - protein, 4 aa, Artificial sequence
  Synthetic
  MISC_FEATURE (2)..(2): Xaa=any amino acid
  MISC_FEATURE (3)..(3): Xaa=D or N
YXXG

SEQ ID NO: 15 - protein, 4 aa, Artificial sequence
  Synthetic
  MISC_FEATURE (2)..(2): Xaa=any amino acid
  MISC_FEATURE (3)..(3): Xaa=D or N
WXXG

SEQ ID NO: 16 - protein, 4 aa, Artificial sequence
  Synthetic
  MISC_FEATURE (2)..(2): Xaa=any amino acid
  MISC_FEATURE (3)..(3): Xaa=D or N
HXXG

SEQ ID NO: 17 - protein, 4 aa, Artificial sequence
  Synthetic
  MISC_FEATURE (2)..(2): Xaa=any amino acid
  MISC_FEATURE (3)..(3): Xaa=D or N
RXXG

SEQ ID NO: 18 - protein, 4 aa, Artificial sequence
  Synthetic
  MISC_FEATURE (2)..(2): Xaa=any amino acid
  MISC_FEATURE (3)..(3): Xaa=D or N
QXXG

SEQ ID NO: 19 - protein, 4 aa, Artificial sequence
  Synthetic
  MISC_FEATURE (2)..(2): Xaa=any amino acid
  MISC_FEATURE (3)..(3): Xaa=D or N
NXXG

SEQ ID NO: 20 - protein, 4 aa, Artificial sequence
  Synthetic
  MISC_FEATURE (2)..(2): Xaa=any amino acid
  MISC_FEATURE (3)..(3): Xaa=D or N
EXXG

SEQ ID NO: 21 - protein, 4 aa, Artificial sequence
  Synthetic
  MISC_FEATURE (2)..(2): Xaa=any amino acid
  MISC_FEATURE (3)..(3): Xaa=D or N
DXXG

SEQ ID NO: 22 - protein, 4 aa, Artificial sequence
  Synthetic
  MISC_FEATURE (2)..(2): Xaa=any amino acid
  MISC_FEATURE (3)..(3): Xaa=D or N
SXXG

SEQ ID NO: 23 - protein, 4 aa, Artificial sequence
  Synthetic
  MISC_FEATURE (2)..(2): Xaa=any amino acid
  MISC_FEATURE (3)..(3): Xaa=D or N
TXXG

SEQ ID NO: 24 - protein, 3 aa, Artificial sequence
  Synthetic
  MISC_FEATURE (1)..(1): Xaa=any amino acid
  MISC_FEATURE (2)..(2): Xaa=D or N
XXG